European Patent Application EP 4 491 631 A1, published January 15, 2025. Title: Anti-PD-1 antibody binding domain. Applicant: Anaveon AG. The sequence listing filed with the application follows.

SEQUENCE LISTING (167 sequences)

SEQ ID NO: 1 - protein, 451 aa, synthetic construct
EVQLVQSGAEVKKPGESLKISCKGSGYAFTNYLIEWVRQMPGKGLEWMGVINPGSGGTNYNEKFKGQVTISADKSISTAYLQWSSLKASDTAMYYCARWRGEGYYAYFDVWGQGTTVTVSSASTKGPSVFPLAPSSKSTSGGTAALGCLVKDYFPEPVTVSWNSGALTSGVHTFPAVLQSSGLYSLSSVVTVPSSSLGTQTYICNVNHKPSNTKVDKRVEPKSCDKTHTCPPCPAPELLGGPSVFLFPPKPKDTLMISRTPEVTCVVVDVSHEDPEVKFNWYVDGVEVHNAKTKPREEQYASTYRVVSVLTVLHQDWLNGKEYKCKVSNKALPAPIEKTISKAKGQPREPQVYTLPPSREEMTKNQVSLTCLVKGFYPSDIAVEWESNGQPENNYKTTPPVLDSDGSFFLYSKLTVDKSRWQQGNVFSCSVMHEALHNHYTQKSLSLSPGK

SEQ ID NO: 2 - protein, 218 aa, synthetic construct
AIRLTQSPSSFSASTGDRVTITCKASQSVDYQGDSYMNWYQQKPGKAPKLLIYAASNLESGVPSRFSGSGSGTDFTLTISSLQSEDFATYYCQQSNEDPYTFGGGTKVEIKRTVAAPSVFIFPPSDEQLKSGTASVVCLLNNFYPREAKVQWKVDNALQSGNSQESVTEQDSKDSTYSLSSTLTLSKADYEKHKVYACEVTHQGLSSPVTKSFNRGEC

SEQ ID NO: 3 - protein, 451 aa, synthetic construct
QVQLVESGGGVVQPGRSLRLSCAASGYTFSSYLIEWVRQAPGKGLEWVAVINPGSGGTNYADSVKGRFTISADKSKNTAYLQMNSLRAEDTAVYYCARWRGDGYYAYFDVWGQGTTVTVSSASTKGPSVFPLAPSSKSTSGGTAALGCLVKDYFPEPVTVSWNSGALTSGVHTFPAVLQSSGLYSLSSVVTVPSSSLGTQTYICNVNHKPSNTKVDKRVEPKSCDKTHTCPPCPAPELLGGPSVFLFPPKPKDTLMISRTPEVTCVVVDVSHEDPEVKFNWYVDGVEVHNAKTKPREEQYNSTYRVVSVLTVLHQDWLNGKEYKCKVSNKALPAPIEKTISKAKGQPREPQVYTLPPSREEMTKNQVSLTCLVKGFYPSDIAVEWESNGQPENNYKTTPPVLDSDGSFFLYSKLTVDKSRWQQGNVFSCSVMHEALHNHYTQKSLSLSPGK

SEQ ID NO: 4 - protein, 218 aa, synthetic construct
EIVLTQSPATLSVSPGERATLSCRASQSVSYDGDSYMNWYQQKPGQAPRLLIYAASNLASGIPARFSGSGSGTEFTLTISSLQSEDAAVYYCQQSNEDPYTFGGGTKVEIKRTVAAPSVFIFPPSDEQLKSGTASVVCLLNNFYPREAKVQWKVDNALQSGNSQESVTEQDSKDSTYSLSSTLTLSKADYEKHKVYACEVTHQGLSSPVTKSFNRGEC

SEQ ID NO: 5 - protein, 153 aa, Homo sapiens
MYRMQLLSCIALSLALVTNSAPTSSSTKKTQLQLEHLLLDLQMILNGINNYKNPKLTRMLTFKFYMPKKATELKHLQCLEEELKPLEEVLNLAQSKNFHLRPRDLISNINVIVLELKGSETTFMCEYADETATIVEFLNRWITFCQSIISTLT

SEQ ID NO: 6 - protein, 134 aa, synthetic construct
MAPTSSSTKKTQLQLEHLLLDLQMILNGINNYKNPKLTRMLTFKFYMPKKATELKHLQCLEEELKPLEEVLNLAQSKNFHLRPRDLISNINVIVLELKGSETTFMCEYADETATIVEFLNRWITFSQSIISTLT

SEQ ID NO: 7 - protein, 133 aa, synthetic construct
APTSSSTKKTQLQLEHLLLDLQMILNGINNYKNPKLTAMLTAKFAMPKKATELKHLQCLEEALKPLEEVLNLAQSKNFHLRPRDLISNINVIVLELKGSETTFMCEYADETATIVEFLNRWITFCQSIISTLT

SEQ ID NO: 8 - protein, 133 aa, synthetic construct
APTSSSTKKTQLQLEHLLLDLQMILNGINNYKNPKLTRMLTAKFAMPKKATELKHLQCLEEELKPLEEVLNGAQSKNFHLRPRDLISNINVIVLELKGSETTFMCEYADETATIVEFLNRWITFCQSIISTLT

SEQ ID NO: 9 - protein, 133 aa, synthetic construct
APTSSSTKKTQLQLEHLLLDLQMILNGINNYKNPKLTRMLTFKFYMPKKATELKHLQCLEEELKPLEEVLNLAQSKNFHFDPRDVVSNINVFVLELKGSETTFMCEYADETATIVEFLNRWITFCQSIISTLT

SEQ ID NO: 10 - protein, 132 aa, synthetic construct
NFHLRPRDLISNINVIVLELKGSETTFMCEYADETATIVEFLNRWITFSQSIISTLTPTSSSTKKTQLQLEHLLLDLQMILNGINNYKNPKLTRMLTFKFYMPKKATELKHLQCLEEELKPLEEVLNLAQSK

SEQ ID NO: 11 - protein, 131 aa, synthetic construct
FHLRPRDLISNINVIVLELKGSETTFMCEYADETATIVEFLNRWITFSQSIISTLTPTSSSTKKTQLQLEHLLLDLQMILNGINNYKNPKLTRMLTFKFYMPKKATELKHLQCLEEELKPLEEVLNLAQSK

SEQ ID NO: 12 - protein, 132 aa, synthetic construct
FYMPKKATELKHLQCLEEELKPLEEVLNLAQSKNFHLRPRDLISNINVIVLELKGSETTFMCEYADETATIVEFLNRWITFSQSIISTLTPTSSSTKKTQLQLEHLLLDLQMILNGINNYKNPKLTRMLTFK

SEQ ID NO: 13 - protein, 132 aa, synthetic construct
ATIVEFLNRWITFCQSIISTLTPTSSSTKKTQLQLEHLLLDLQMILNGINNYKNPKLTRMLTFKFYMPKKATELKHLQCLEEELKPLEEVLNLAQSKNFHLRPRDLISNINVIVLELKGSETTFMCEYADET

SEQ ID NO: 14-16 - skipped (3 entries)

SEQ ID NO: 17 - protein, 4 aa, synthetic construct
GGGG

SEQ ID NO: 18 - protein, 5 aa, synthetic construct
GGGGS

SEQ ID NO: 19 - protein, 6 aa, synthetic construct
GGGGSG

SEQ ID NO: 20 - protein, 7 aa, synthetic construct
GGGGSGG

SEQ ID NO: 21 - protein, 13 aa, synthetic construct
GGGGSGGGGSGGG

SEQ ID NO: 22 - protein, 14 aa, synthetic construct
GGGGSGGGGSGGGG

SEQ ID NO: 23 - protein, 19 aa, synthetic construct
GGGGSGGGGSGGGGSGGGG

SEQ ID NO: 24 - protein, 20 aa, synthetic construct
GGGGSGGGGSGGGGSGGGGS

SEQ ID NO: 25 - protein, 242 aa, synthetic construct
AIRLTQSPSSFSASTGDRVTITCKASQSVDYNFHLRPRDLISNINVIVLELKGSETTFMCEYADETATIVEFLNRWITFSQSIISTLTPTSSSTKKTQLQLEHLLLDLQMILNGINNYKNPKLTRMLTFKFYMPKKATELKHLQCLEEELKPLEEVLNLAQSKGDSYMNWYQQKPGKAPKLLIYAASNLESGVPSRFSGSGSGTDFTLTISSLQSEDFATYYCQQSNEDPYTFGGGTKVEIK

SEQ ID NO: 26 - protein, 246 aa, synthetic construct
AIRLTQSPSSFSASTGDRVTITCKASQSVDYGGNFHLRPRDLISNINVIVLELKGSETTFMCEYADETATIVEFLNRWITFSQSIISTLTPTSSSTKKTQLQLEHLLLDLQMILNGINNYKNPKLTRMLTFKFYMPKKATELKHLQCLEEELKPLEEVLNLAQSKGGGDSYMNWYQQKPGKAPKLLIYAASNLESGVPSRFSGSGSGTDFTLTISSLQSEDFATYYCQQSNEDPYTFGGGTKVEIK

SEQ ID NO: 27 - protein, 248 aa, synthetic construct
AIRLTQSPSSFSASTGDRVTITCKASQSVDYGGGNFHLRPRDLISNINVIVLELKGSETTFMCEYADETATIVEFLNRWITFSQSIISTLTPTSSSTKKTQLQLEHLLLDLQMILNGINNYKNPKLTRMLTFKFYMPKKATELKHLQCLEEELKPLEEVLNLAQSKGGGGDSYMNWYQQKPGKAPKLLIYAASNLESGVPSRFSGSGSGTDFTLTISSLQSEDFATYYCQQSNEDPYTFGGGTKVEIK

SEQ ID NO: 28 - protein, 250 aa, synthetic construct
AIRLTQSPSSFSASTGDRVTITCKASQSVDYGGGGNFHLRPRDLISNINVIVLELKGSETTFMCEYADETATIVEFLNRWITFSQSIISTLTPTSSSTKKTQLQLEHLLLDLQMILNGINNYKNPKLTRMLTFKFYMPKKATELKHLQCLEEELKPLEEVLNLAQSKGGGGSDSYMNWYQQKPGKAPKLLIYAASNLESGVPSRFSGSGSGTDFTLTISSLQSEDFATYYCQQSNEDPYTFGGGTKVEIK

SEQ ID NO: 29 - protein, 254 aa, synthetic construct
AIRLTQSPSSFSASTGDRVTITCKASQSVDYGGGGSGNFHLRPRDLISNINVIVLELKGSETTFMCEYADETATIVEFLNRWITFSQSIISTLTPTSSSTKKTQLQLEHLLLDLQMILNGINNYKNPKLTRMLTFKFYMPKKATELKHLQCLEEELKPLEEVLNLAQSKGGGGSGGDSYMNWYQQKPGKAPKLLIYAASNLESGVPSRFSGSGSGTDFTLTISSLQSEDFATYYCQQSNEDPYTFGGGTKVEIK

SEQ ID NO: 30 - protein, 268 aa, synthetic construct
AIRLTQSPSSFSASTGDRVTITCKASQSVDYGGGGSGGGGSGGGNFHLRPRDLISNINVIVLELKGSETTFMCEYADETATIVEFLNRWITFSQSIISTLTPTSSSTKKTQLQLEHLLLDLQMILNGINNYKNPKLTRMLTFKFYMPKKATELKHLQCLEEELKPLEEVLNLAQSKGGGGSGGGGSGGGGDSYMNWYQQKPGKAPKLLIYAASNLESGVPSRFSGSGSGTDFTLTISSLQSEDFATYYCQQSNEDPYTFGGGTKVEIK

SEQ ID NO: 31 - protein, 280 aa, synthetic construct
AIRLTQSPSSFSASTGDRVTITCKASQSVDYGGGGSGGGGSGGGGSGGGGNFHLRPRDLISNINVIVLELKGSETTFMCEYADETATIVEFLNRWITFSQSIISTLTPTSSSTKKTQLQLEHLLLDLQMILNGINNYKNPKLTRMLTFKFYMPKKATELKHLQCLEEELKPLEEVLNLAQSKGGGGSGGGGSGGGGSGGGGSDSYMNWYQQKPGKAPKLLIYAASNLESGVPSRFSGSGSGTDFTLTISSLQSEDFATYYCQQSNEDPYTFGGGTKVEIK

SEQ ID NO: 32 - protein, 242 aa, synthetic construct
EIVLTQSPATLSVSPGERATLSCRASQSVSYNFHLRPRDLISNINVIVLELKGSETTFMCEYADETATIVEFLNRWITFSQSIISTLTPTSSSTKKTQLQLEHLLLDLQMILNGINNYKNPKLTRMLTFKFYMPKKATELKHLQCLEEELKPLEEVLNLAQSKGDSYMNWYQQKPGQAPRLLIYAASNLASGIPARFSGSGSGTEFTLTISSLQSEDAAVYYCQQSNEDPYTFGGGTKVEIK

SEQ ID NO: 33 - protein, 246 aa, synthetic construct
EIVLTQSPATLSVSPGERATLSCRASQSVSYGGNFHLRPRDLISNINVIVLELKGSETTFMCEYADETATIVEFLNRWITFSQSIISTLTPTSSSTKKTQLQLEHLLLDLQMILNGINNYKNPKLTRMLTFKFYMPKKATELKHLQCLEEELKPLEEVLNLAQSKGGGDSYMNWYQQKPGQAPRLLIYAASNLASGIPARFSGSGSGTEFTLTISSLQSEDAAVYYCQQSNEDPYTFGGGTKVEIK

SEQ ID NO: 34 - protein, 248 aa, synthetic construct
EIVLTQSPATLSVSPGERATLSCRASQSVSYGGGNFHLRPRDLISNINVIVLELKGSETTFMCEYADETATIVEFLNRWITFSQSIISTLTPTSSSTKKTQLQLEHLLLDLQMILNGINNYKNPKLTRMLTFKFYMPKKATELKHLQCLEEELKPLEEVLNLAQSKGGGGDSYMNWYQQKPGQAPRLLIYAASNLASGIPARFSGSGSGTEFTLTISSLQSEDAAVYYCQQSNEDPYTFGGGTKVEIK

SEQ ID NO: 35 - protein, 254 aa, synthetic construct
EIVLTQSPATLSVSPGERATLSCRASQSVSYGGGGSGNFHLRPRDLISNINVIVLELKGSETTFMCEYADETATIVEFLNRWITFSQSIISTLTPTSSSTKKTQLQLEHLLLDLQMILNGINNYKNPKLTRMLTFKFYMPKKATELKHLQCLEEELKPLEEVLNLAQSKGGGGSGGDSYMNWYQQKPGQAPRLLIYAASNLASGIPARFSGSGSGTEFTLTISSLQSEDAAVYYCQQSNEDPYTFGGGTKVEIK

SEQ ID NO: 36 - protein, 268 aa, synthetic construct
EIVLTQSPATLSVSPGERATLSCRASQSVSYGGGGSGGGGSGGGNFHLRPRDLISNINVIVLELKGSETTFMCEYADETATIVEFLNRWITFSQSIISTLTPTSSSTKKTQLQLEHLLLDLQMILNGINNYKNPKLTRMLTFKFYMPKKATELKHLQCLEEELKPLEEVLNLAQSKGGGGSGGGGSGGGGDSYMNWYQQKPGQAPRLLIYAASNLASGIPARFSGSGSGTEFTLTISSLQSEDAAVYYCQQSNEDPYTFGGGTKVEIK

SEQ ID NO: 37 - protein, 240 aa, synthetic construct
DIQMTQSPSSVSASVGDRVTITCSASQGISGNFHLRPRDLISNINVIVLELKGSETTFMCEYADETATIVEFLNRWITFSQSIISTLTPTSSSTKKTQLQLEHLLLDLQMILNGINNYKNPKLTRMLTFKFYMPKKATELKHLQCLEEELKPLEEVLNLAQSKGDLNWYQQKPGKAPKLLIYHTSSLHSGVPSRFSGSGSGTDFTLTISSLQPEDFATYYCQYYSKDLLTFGGGTKLEIK

SEQ ID NO: 38 - protein, 244 aa, synthetic construct
DIQMTQSPSSVSASVGDRVTITCSASQGISGGGNFHLRPRDLISNINVIVLELKGSETTFMCEYADETATIVEFLNRWITFSQSIISTLTPTSSSTKKTQLQLEHLLLDLQMILNGINNYKNPKLTRMLTFKFYMPKKATELKHLQCLEEELKPLEEVLNLAQSKGGGDLNWYQQKPGKAPKLLIYHTSSLHSGVPSRFSGSGSGTDFTLTISSLQPEDFATYYCQYYSKDLLTFGGGTKLEIK

SEQ ID NO: 39 - protein, 246 aa, synthetic construct
DIQMTQSPSSVSASVGDRVTITCSASQGISGGGGNFHLRPRDLISNINVIVLELKGSETTFMCEYADETATIVEFLNRWITFSQSIISTLTPTSSSTKKTQLQLEHLLLDLQMILNGINNYKNPKLTRMLTFKFYMPKKATELKHLQCLEEELKPLEEVLNLAQSKGGGGDLNWYQQKPGKAPKLLIYHTSSLHSGVPSRFSGSGSGTDFTLTISSLQPEDFATYYCQYYSKDLLTFGGGTKLEIK

SEQ ID NO: 40 - protein, 252 aa, synthetic construct
DIQMTQSPSSVSASVGDRVTITCSASQGISGGGGGSGNFHLRPRDLISNINVIVLELKGSETTFMCEYADETATIVEFLNRWITFSQSIISTLTPTSSSTKKTQLQLEHLLLDLQMILNGINNYKNPKLTRMLTFKFYMPKKATELKHLQCLEEELKPLEEVLNLAQSKGGGGSGGDLNWYQQKPGKAPKLLIYHTSSLHSGVPSRFSGSGSGTDFTLTISSLQPEDFATYYCQYYSKDLLTFGGGTKLEIK

SEQ ID NO: 41 - protein, 266 aa, synthetic construct
DIQMTQSPSSVSASVGDRVTITCSASQGISGGGGGSGGGGSGGGNFHLRPRDLISNINVIVLELKGSETTFMCEYADETATIVEFLNRWITFSQSIISTLTPTSSSTKKTQLQLEHLLLDLQMILNGINNYKNPKLTRMLTFKFYMPKKATELKHLQCLEEELKPLEEVLNLAQSKGGGGSGGGGSGGGGDLNWYQQKPGKAPKLLIYHTSSLHSGVPSRFSGSGSGTDFTLTISSLQPEDFATYYCQYYSKDLLTFGGGTKLEIK

SEQ ID NO: 42 - protein, 111 aa, synthetic construct
AIRLTQSPSSFSASTGDRVTITCKASQSVDYQGDSYMNWYQQKPGKAPKLLIYAASNLESGVPSRFSGSGSGTDFTLTISSLQSEDFATYYCQQSNEDPYTFGGGTKVEIK

SEQ ID NO: 43 - protein, 121 aa, synthetic construct
EVQLVQSGAEVKKPGESLKISCKGSGYAFTNYLIEWVRQMPGKGLEWMGVINPGSGGTNYNEKFKGQVTISADKSISTAYLQWSSLKASDTAMYYCARWRGEGYYAYFDVWGQGTTVTVSS

SEQ ID NO: 44 - protein, 121 aa, synthetic construct
QVQLVESGGGVVQPGRSLRLSCAASGYTFSSYLIEWVRQAPGKGLEWVAVINPGSGGTNYADSVKGRFTISADKSKNTAYLQMNSLRAEDTAVYYCARWRGDGYYAYFDVWGQGTTVTVSS

SEQ ID NO: 45 - protein, 117 aa, synthetic construct
EVQLVQSGAEVKKPGESLKISCKGSGYSFTNFYIHWVRQAPGQRLEWMGSIYPNYGDTAYNQKFKDRFVFSLDTSVSTAYLQISSLKAEDTAVYYCARGYSYAMDYWGQGTTVTVSS

SEQ ID NO: 46 - protein, 258 aa, synthetic construct
EVQLVQSGAEVKKPGESLKISCKGSGYAFTNYLIEWVRQMPGKGLEWMGVINPGSGGTNYNEKFKGQVTISADKSISTAYLQWSSLKASDTAMYYCARWRGEGGGFHLRPRDLISNINVIVLELKGSETTFMCEYADETATIVEFLNRWITFSQSIISTLTPTSSSTKKTQLQLEHLLLDLQMILNGINNYKNPKLTRMLTFKFYMPKKATELKHLQCLEEELKPLEEVLNLAQSKGGGGYYAYFDVWGQGTTVTVSS

SEQ ID NO: 47 - protein, 258 aa, synthetic construct
EVQLVQSGAEVKKPGESLKISCKGSGYAFTNYLIEWVRQMPGKGLEWMGVINPGGGFYMPKKATELKHLQCLEEELKPLEEVLNLAQSKNFHLRPRDLISNINVIVLELKGSETTFMCEYADETATIVEFLNRWITFCQSIISTLTPTSSSTKKTQLQLEHLLLDLQMILNGINNYKNPKLTRMLTFKGGGSGGTNYNEKFKGQVTISADKSISTAYLQWSSLKASDTAMYYCARWRGEGYYAYFDVWGQGTTVTVSS

SEQ ID NO: 48 - protein, 330 aa, synthetic construct
ASTKGPSVFPLAPSSKSTSGGTAALGCLVKDYFPEPVTVSWNSGALTSGVHTFPAVLQSSGLYSLSSVVTVPSSSLGTQTYICNVNHKPSNTKVDKRVEPKSCDKTHTCPPCPAPELLGGPSVFLFPPKPKDTLMISRTPEVTCVVVDVSHEDPEVKFNWYVDGVEVHNAKTKPREEQYASTYRVVSVLTVLHQDWLNGKEYKCKVSNKALPAPIEKTISKAKGQPREPQVYTLPPSREEMTKNQVSLTCLVKGFYPSDIAVEWESNGQPENNYKTTPPVLDSDGSFFLYSKLTVDKSRWQQGNVFSCSVMHEALHNHYTQKSLSLSPGK

SEQ ID NO: 49 - protein, 107 aa, synthetic construct [sequence omitted]

SEQ ID NO: 50 - protein, 111 aa, synthetic construct
EIVLTQSPATLSVSPGERATLSCRASQSVSYDGDSYMNWYQQKPGQAPRLLIYAASNLASGIPARFSGSGSGTEFTLTISSLQSEDAAVYYCQQSNEDPYTFGGGTKVEIK

SEQ ID NO: 51 - protein, 451 aa, synthetic construct; identical to SEQ ID NO: 1

SEQ ID NO: 52 - protein, 355 aa, synthetic construct
AIRLTQSPSSFSASTGDRVTITCKASQSVDYGGGNFHLRPRDLISNINVIVLELKGSETTFMCEYADETATIVEFLNRWITFSQSIISTLTPTSSSTKKTQLQLEHLLLDLQMILNGINNYKNPKLTRMLTFKFYMPKKATELKHLQCLEEELKPLEEVLNLAQSKGGGGDSYMNWYQQKPGKAPKLLIYAASNLESGVPSRFSGSGSGTDFTLTISSLQSEDFATYYCQQSNEDPYTFGGGTKVEIKRTVAAPSVFIFPPSDEQLKSGTASVVCLLNNFYPREAKVQWKVDNALQSGNSQESVTEQDSKDSTYSLSSTLTLSKADYEKHKVYACEVTHQGLSSPVTKSFNRGEC

SEQ ID NO: 53 - protein, 447 aa, synthetic construct
QVQLVQSGAEVKKPGASVKVSCKASGYTFTNFYIHWVRQAPGQGLEWMGSIYPNYGDTAYNQKFKDRVTMTTDTSTSTAYMELRSLRSDDTAVYYCARGYSYAMDYWGQGTTVTVSSASTKGPSVFPLAPSSKSTSGGTAALGCLVKDYFPEPVTVSWNSGALTSGVHTFPAVLQSSGLYSLSSVVTVPSSSLGTQTYICNVNHKPSNTKVDKKVEPKSCDKTHTCPPCPAPELLGGPSVFLFPPKPKDTLMISRTPEVTCVVVDVSHEDPEVKFNWYVDGVEVHNAKTKPREEQYNSTYRVVSVLTVLHQDWLNGKEYKCKVSNKALPAPIEKTISKAKGQPREPQVYTLPPSRDELTKNQVSLTCLVKGFYPSDIAVEWESNGQPENNYKTTPPVLDSDGSFFLYSKLTVDKSRWQQGNVFSCSVMHEALHNHYTQKSLSLSPGK

SEQ ID NO: 54 - protein, 214 aa, synthetic construct
DIQMTQSPSSVSASVGDRVTITCSASQGISGDLNWYQQKPGKAPKLLIYHTSSLHSGVPSRFSGSGSGTDFTLTISSLQPEDFATYYCQYYSKDLLTFGGGTKLEIKRTVAAPSVFIFPPSDEQLKSGTASVVCLLNNFYPREAKVQWKVDNALQSGNSQESVTEQDSKDSTYSLSSTLTLSKADYEKHKVYACEVTHQGLSSPVTKSFNRGEC

SEQ ID NO: 55 - protein, 117 aa, synthetic construct
QVQLVQSGAEVKKPGASVKVSCKASGYTFTNFYIHWVRQAPGQGLEWMGSIYPNYGDTAYNQKFKDRVTMTVDTSTSTAYMELRSLRSDDTAVYYCARGYSYAMDYWGQGTTVTVSS

SEQ ID NO: 56 - protein, 107 aa, synthetic construct
DIQMTQSPSSVSASVGDRVTITCSASQGISGDLNWYQQKPGKAPKLLIYHTSSLHSGVPSRFSGSGSGTDFTLTISSLQPEDFATYYCQYYSKDLLTFGGGTKLEIK

SEQ ID NO: 57 - protein, 117 aa, synthetic construct
QVQLVQSGAEVKKPGASVKVSCKASGYTFTNFYIHWVRQAPGQGLEWMGSIYPNYGFTAYNQKFKDRVTMTVDTSTSTAYMELRSLRSDDTAVYYCARGYSYAMDYWGQGTTVTVSS

SEQ ID NO: 58 - protein, 107 aa, synthetic construct
DIQMTQSPSSVSASVGDRVTITCSASQGIWGDLNWYQQKPGKAPKLLIYHTSQLHSDVPSRFSGSGSGTDFTLTISSLQPEDFATYYCQGYSKDLLTFGGGTKLEIK

SEQ ID NO: 59 - protein, 117 aa, synthetic construct
QVQLVQSGAEVKKPGASVKVSCKASGYTFTNFYIHWVRQAPGQGLEWMGRIYPNYGFTAYNQKFKDRVTMTVDTSTSTAYMELRSLRSDDTAVYYCARGYSYAMDYWGQGTTVTVSS

SEQ ID NO: 60 - protein, 107 aa, synthetic construct
DIQMTQSPSSVSASVGDRVTITCSASQGIYGDLNWYQQKPGKAPKLLIYHTSSLHSGVPSRFSGSGSGTDFTLTISSLQPEDFATYYCQAYSKDLLTFGGGTKLEIK

SEQ ID NO: 61 - protein, 117 aa, synthetic construct
QVQLVQSGAEVKKPGASVKVSCKASGYTFTNFYIHWVRQAPGQGLEWMGRIYPNYGITAYNQKFKDRVTMTVDTSTSTAYMELRSLRSDDTAVYYCARGYSYAMDYWGQGTTVTVSS

SEQ ID NO: 62 - protein, 107 aa, synthetic construct
DIQMTQSPSSVSASVGDRVTITCSASQGISGDLNWYQQKPGKAPKLLIYHTSQRHSDVPSRFSGSGSGTDFTLTISSLQPEDFATYYCQGYSKDLLTFGGGTKLEIK

SEQ ID NO: 63 - protein, 117 aa, synthetic construct; identical to SEQ ID NO: 61

SEQ ID NO: 64 - protein, 107 aa, synthetic construct
DIQMTQSPSSVSASVGDRVTITCSASQGISGDLNWYQQKPGKAPKLLIYHTSSRHSGVPSRFSGSGSGTDFTLTISSLQPEDFATYYCQGYSKDLLTFGGGTKLEIK

SEQ ID NO: 65 - protein, 117 aa, synthetic construct; identical to SEQ ID NO: 61

SEQ ID NO: 66 - protein, 107 aa, synthetic construct
DIQMTQSPSSVSASVGDRVTITCSASQGIYGDLNWYQQKPGKAPKLLIYHTSSRHSGVPSRFSGSGSGTDFTLTISSLQPEDFATYYCQAYSKDLLTFGGGTKLEIK

SEQ ID NO: 67 - protein, 117 aa, synthetic construct
QVQLVQSGAEVKKPGASVKVSCKASGYTFTNFYIHWVRQAPGQGLEWMGSIYPNYGITAYNQKFKDRVTMTVDTSTSTAYMELRSLRSDDTAVYYCARGYSYAMDYWGQGTTVTVSS

SEQ ID NO: 68 - protein, 107 aa, synthetic construct
DIQMTQSPSSVSASVGDRVTITCSASQGISGDLNWYQQKPGKAPKLLIYHTSQLHSDVPSRFSGSGSGTDFTLTISSLQPEDFATYYCQGYSKDLLTFGGGTKLEIK

SEQ ID NO: 69 - protein, 114 aa, synthetic construct
QVQLVQSGAEVKKPGASVKVSCKASGYDFTSHWMHWVRQAPGQGLEWMGAIDPSDSYTNYNQKFKGRVTMTTDTSTSTAYMELRSLRSDDTAVYYCARSPFDYWGQGTTVTVSS

SEQ ID NO: 70 - protein, 107 aa, synthetic construct
DIQMTQSPSSLSASVGDRVTITCKASQDVSTAVAWYQQKPGKAPKLLIYSASYRYTGVPSRFSGSGSGTDFTFTISSLQPEDIATYYCQQHYSFPFTFGQGTKLEIK

SEQ ID NO: 71 - protein, 115 aa, synthetic construct
EVQLLESGGGLVQPGGSLRLSCAASGFTFSINAMTWVRQAPGKGLEWVSTISGSGFSTYYADSLKGRFTISRDNSKNTLYLQMNSLRAEDTAVYYCAKEVYGDYWGQGTLVTVSS

SEQ ID NO: 72 - protein, 110 aa, synthetic construct
RSVLTQPPSASGTPGQRVSISCSGNSSNIGSNSVFWYQQLPGTAPKLLIYSNNQRPSGVPDRFSGSKSGTSASLAISGLRSEDEADYYCAAWDDSLSIWVFGGGTKLTVL

SEQ ID NO: 73 - protein, 115 aa, synthetic construct
EVQLLESGGGLVQPGGSLRLSCAASGFTFSISAMTWVRQAPGKGLEWVSTISGSGGSTYYSDSVKGRFTISRDNSKNTLYLQINSLRADDTAVYYCAKEVYGDYWGQGTLVTVSS

SEQ ID NO: 74 - protein, 110 aa, synthetic construct
QSILTQPPSASGTPGQRVTISCSGSSSNIGSNSVFWYQQLPGTAPKLLIFSNNQRPSGVPDRFSGSKSGTSASLAISGLRSEDEADYCCAAWDDSLSGWIFGGGTKLTVL

SEQ ID NO: 75 - protein, 115 aa, synthetic construct
EVQLLESGGNLVQPGGSLRLSCAASGFTFSTYAMSWVRQAPGKGLEWVSTISGTGYSTYFADSVKGRFTISRDNSKNTLFLQMNSLRAEDTAVYYCAKEVYGDYWGQGTLVTVSS

SEQ ID NO: 76 - protein, 110 aa, synthetic construct
QSVLTQPPSASGTPGQRVTISCSGRSSNIGSNSIFWYQQLPGTAPKLLIYSNNQRPSGVPDRFSGSKSGTSASLAISGLRSEDETDYYCAAWDDSLSGWVFGGGTKLTVL

SEQ ID NO: 77 - protein, 117 aa, synthetic construct
EVLLVESGGGLVQPGGSLRLSCAASGFTFSSYSMNWVRQAPGKGLEWVSFISSSSPTLYYADSVKGRFTISRDNAKNSLYLQMNSLRDEDTAVYYCARQGLTPFDYWGQGTLVTVSS

SEQ ID NO: 78 - protein, 107 aa, synthetic construct
EIVMTQSPATLSVFPGERATLSCRASQSVSSYLAWYQQKPGQAPRLLIYGASTRATGIPARVSGSGSGTEFILTISSLQSEDFAVYYCQQYNNWPYTFGQGTKLEIK

SEQ ID NO: 79 - protein, 113 aa, synthetic construct
QVQLVESGGGVGQPGRSLRLSCAASGFTFSNYGMHWVRQAPGKGLEWVAVIWYDGSKKYYADSVKGRFTISRDNSKNTLYLQMNSLRVEDTAVYYCVGNSGHWGQGTLVTVSS

SEQ ID NO: 80 - protein, 113 aa, synthetic construct
DIVMTQTPLSLPVTPGEPASISCRSSQSLLDSDDGNTYLDWYLQKPGQSPQLLIYTLSYRASGVPDRFSGSGSGTDFTLKISRVEAEDVGVYYCMQCIEFPHTFGGGTKVEIK

SEQ ID NO: 81 - protein, 117 aa, synthetic construct
EVQLVESGGGLVQPGGSLRLSCAASGFTFSSYSMNWVRQAPGKGLQWVSYITSSSNTMYYADSVKGRFTISRDNAKNSLYLQMNSLRDEDTAVYYCASIVGAPFDYWGQGTLVTVSS

SEQ ID NO: 82 - protein, 107 aa, synthetic construct
EIVMTQSPATLSVSPGERATLSCRASQSVSSSLAWYQQKPGQAPRLLIYGASTRATGIPARFSGSGSGTEFTLTISSLQSEDFAAYYCQQYNNWPFTFGPGTKVDIK

SEQ ID NO: 83 - protein, 127 aa, synthetic construct
QVQLVQSGAEVKKPGASVKVSCKASGYTFTSYFMHWVRQAPGQGLEWMGLINPDGGNTDYAQKFQGRVTMTRDTSTSTVYMELSSLRSEDTAVYYCARDGNYYDSSGYYYPDAFDIWGQGTMVTVSS

SEQ ID NO: 84 - protein, 108 aa, synthetic construct
SSELTQDPAVSVALGQTVRITCQGDSLRRFYASWYQQKPGQAPVIVIYGKDNRPSGTPDRFSGSTSGNTASLTITGAQAEDEADYYCNSRDSSGTHVVFGGGTKLTVL

SEQ ID NO: 85 - protein, 115 aa, synthetic construct; identical to SEQ ID NO: 71

SEQ ID NO: 86 - protein, 110 aa, synthetic construct
RSVLTQPPSASGTPGQRVSISCSGASSNIGSQSVFWYQQLPGTAPKLLIYSNNQRPSGVPDRFSGSKSGTSASLAISGLRSEDEADYYCAAWDDSLSIWVFGGGTKLTVL

SEQ ID NO: 87 - protein, 110 aa, synthetic construct
RSVLTQPPSASGTPGQRVSISCSGASSNIGSSSVFWYQQLPGTAPKLLIYSNNQRPSGVPDRFSGSKSGTSASLAISGLRSEDEADYYCAAWDDSLSIWVFGGGTKLTVL

SEQ ID NO: 88 - protein, 449 aa, synthetic construct
EVQLLESGGGLVQPGGSLRLSCAASGFTFSINAMTWVRQAPGKGLEWVSTISGSGFSTYYADSLKGRFTISRDNSKNTLYLQMNSLRAEDTAVYYCAKEVYGDYWGQGTLVTVSSASVAAPSVFIFPPSDEQLKSGTASVVCLLNNFYPREAKVQWKVDNALQSGNSQESVTEQDSKDSTYSLSSTLTLSKADYEKHKVYACEVTHQGLSSPVTKSFNRGECDKTHTCPPCPAPEAAGGPSVFLFPPKPKDTLMISRTPEVTCVVVDVSHEDPEVKFNWYVDGVEVHNAKTKPREEQYNSTYRVVSVLTVLHQDWLNGKEYKCKVSNKALAAPIEKTISKAKGQPREPQVYTLPPSREEMTKNQVSLTCLVKGFYPSDIAVEWESNGQPENNYKTTPPVLDSDGSFFLTSKLTVDKSRWQQGNVFSCSVMHEALHNHYTQKSLSLSPGK

SEQ ID NO: 89 - protein, 215 aa, synthetic construct
RSVLTQPPSASGTPGQRVSISCSGASSNIGSQSVFWYQQLPGTAPKLLIYSNNQRPSGVPDRFSGSKSGTSASLAISGLRSEDEADYYCAAWDDSLSIWVFGGGTKLTVLSSASTKGPSVFPLAPSSKSTSGGTAALGCLVKDYFPEPVTVSWNSGALTSGVHTFPAVLQSSGLYSLSSVVTVPSSSLGTQTYICNVNHKPSNTKVDKRVEPKSC

SEQ ID NO: 90 - protein, 451 aa, synthetic construct
EVQLVQSGAEVKKPGESLKISCKGSGYAFTNYLIEWVRQMPGKGLEWMGVINPGSGGTNYNEKFKGQVTISADKSISTAYLQWSSLKASDTAMYYCARWRGEGYYAYFDVWGQGTTVTVSSASTKGPSVFPLAPSSKSTSGGTAALGCLVKDYFPEPVTVSWNSGALTSGVHTFPAVLQSSGLYSLSSVVTVPSSSLGTQTYICNVNHKPSNTKVDKRVEPKSCDKTHTCPPCPAPEAAGGPSVFLFPPKPKDTLMISRTPEVTCVVVDVSHEDPEVKFNWYVDGVEVHNAKTKPREEQYNSTYRVVSVLTVLHQDWLNGKEYKCKVSNKALAAPIEKTISKAKGQPREPQVYTLPPSREEMTKNQVSLYCLVKGFYPSDIAVEWESNGQPENNYKTTPPVLDSDGSFFLYSKLTVDKSRWQQGNVFSCSVMHEALHNHYTQKSLSLSPGK

SEQ ID NO: 91 - protein, 110 aa, synthetic construct
RSVLTQPPSASGTPGQRVSISCSGASSNIGSNAVFWYQQLPGTAPKLLIYSNNQRPSGVPDRFSGSKSGTSASLAISGLRSEDEADYYCAAWDDSLSIWVFGGGTKLTVL

SEQ ID NO: 92 - protein, 449 aa, synthetic construct; identical to SEQ ID NO: 88

SEQ ID NO: 93 - protein, 215 aa, synthetic construct
RSVLTQPPSASGTPGQRVSISCSGASSNIGSSSVFWYQQLPGTAPKLLIYSNNQRPSGVPDRFSGSKSGTSASLAISGLRSEDEADYYCAAWDDSLSIWVFGGGTKLTVLSSASTKGPSVFPLAPSSKSTSGGTAALGCLVKDYFPEPVTVSWNSGALTSGVHTFPAVLQSSGLYSLSSVVTVPSSSLGTQTYICNVNHKPSNTKVDKRVEPKSC

SEQ ID NO: 94 - protein, 445 aa, synthetic construct
EVQLLESGGGLVQPGGSLRLSCAASGFTFSINAMTWVRQAPGKGLEWVSTISGSGFSTYYADSLKGRFTISRDNSKNTLYLQMNSLRAEDTAVYYCAKEVYGDYWGQGTLVTVSSASTKGPSVFPLAPSSKSTSGGTAALGCLVKDYFPEPVTVSWNSGALTSGVHTFPAVLQSSGLYSLSSVVTVPSSSLGTQTYICNVNHKPSNTKVDKRVEPKSCDKTHTCPPCPAPEAAGGPSVFLFPPKPKDTLMISRTPEVTCVVVDVSHEDPEVKFNWYVDGVEVHNAKTKPREEQYNSTYRVVSVLTVLHQDWLNGKEYKCKVSNKALAAPIEKTISKAKGQPREPQVYTLPPSREEMTKNQVSLTCLVKGFYPSDIAVEWESNGQPENNYKTTPPVLDSDGSFFLTSKLTVDKSRWQQGNVFSCSVMHEALHNHYTQKSLSLSPGK

SEQ ID NO: 95 - protein, 216 aa, synthetic construct
RSVLTQPPSASGTPGQRVSISCSGASSNIGSQSVFWYQQLPGTAPKLLIYSNNQRPSGVPDRFSGSKSGTSASLAISGLRSEDEADYYCAAWDDSLSIWVFGGGTKLTVLGQPKAAPSVTLFPPSSEELQANKATLVCLISDFYPGAVTVAWKADSSPVKAGVETTTPSKQSNNKYAASSYLSLTPEQWKSHRSYSCQVTHEGSTVEKTVAPTECS

SEQ ID NO: 96 - protein, 839 aa, synthetic construct
AIRLTQSPSSFSASTGDRVTITCKASQSVDYGGGNFHLRPRDLISNINVIVLELKGSETTFMCEYADETATIVEFLNRWITFSQSIISTLTPTSSSTKKTQLQLEHLLLDLQMILNGINNYKNPKLTRMLTFKFYMPKKATELKHLQCLEEELKPLEEVLNLAQSKGGGGDSYMNWYQQKPGKAPKLLIYAASNLESGVPSRFSGSGSGTDFTLTISSLQSEDFATYYCQQSNEDPYTFGGGTKVEIKGGGGSGGGGSGGGGSEVQLVQSGAEVKKPGESLKISCKGSGYAFTNYLIEWVRQMPGKGLEWMGVINPGSGGTNYNEKFKGQVTISADKSISTAYLQWSSLKASDTAMYYCARWRGEGYYAYFDVWGQGTTVTVSSGGGGSGGGGSEVQLLESGGGLVQPGGSLRLSCAASGFTFSINAMTWVRQAPGKGLEWVSTISGSGFSTYYADSLKGRFTISRDNSKNTLYLQMNSLRAEDTAVYYCAKEVYGDYWGQGTLVTVSSASTKGPSVFPLAPSSKSTSGGTAALGCLVKDYFPEPVTVSWNSGALTSGVHTFPAVLQSSGLYSLSSVVTVPSSSLGTQTYICNVNHKPSNTKVDKRVEPKSCDKTHTCPPCPAPEAAGGPSVFLFPPKPKDTLMISRTPEVTCVVVDVSHEDPEVKFNWYVDGVEVHNAKTKPREEQYNSTYRVVSVLTVLHQDWLNGKEYKCKVSNKALAAPIEKTISKAKGQPREPQVYTLPPSREEMTKNQVSLYCLVKGFYPSDIAVEWESNGQPENNYKTTPPVLDSDGSFFLYSKLTVDKSRWQQGNVFSCSVMHEALHNHYTQKSLSLSPGK

SEQ ID NO: 97 - protein, 445 aa, synthetic construct; identical to SEQ ID NO: 94

SEQ ID NO: 98 - protein, 216 aa, synthetic construct
RSVLTQPPSASGTPGQRVSISCSGASSNIGSSSVFWYQQLPGTAPKLLIYSNNQRPSGVPDRFSGSKSGTSASLAISGLRSEDEADYYCAAWDDSLSIWVFGGGTKLTVLGQPKAAPSVTLFPPSSEELQANKATLVCLISDFYPGAVTVAWKADSSPVKAGVETTTPSKQSNNKYAASSYLSLTPEQWKSHRSYSCQVTHEGSTVEKTVAPTECS

SEQ ID NO: 99 - protein, 839 aa, synthetic construct; identical to SEQ ID NO: 96

SEQ ID NO: 100 - protein, 451 aa, synthetic construct; identical to SEQ ID NO: 90

SEQ ID NO: 101 - protein, 451 aa, synthetic construct
QVQLVQSGAEVKKPGASVKVSCKASGYTFTNFYIHWVRQAPGQGLEWMGRIYPNYGITAYNQKFKDRVTMTVDTSTSTAYMELRSLRSDDTAVYYCARGYSYAMDYWGQGTTVTVSSASVAAPSVFIFPPSDEQLKSGTASVVCLLNNFYPREAKVQWKVDNALQSGNSQESVTEQDSKDSTYSLSSTLTLSKADYEKHKVYACEVTHQGLSSPVTKSFNRGECDKTHTCPPCPAPEAAGGPSVFLFPPKPKDTLMISRTPEVTCVVVDVSHEDPEVKFNWYVDGVEVHNAKTKPREEQYNSTYRVVSVLTVLHQDWLNGKEYKCKVSNKALAAPIEKTISKAKGQPREPQVYTLPPSREEMTKNQVSLTCLVKGFYPSDIAVEWESNGQPENNYKTTPPVLDSDGSFFLTSKLTVDKSRWQQGNVFSCSVMHEALHNHYTQKSLSLSPGK

SEQ ID NO: 102 - protein, 212 aa, synthetic construct
DIQMTQSPSSVSASVGDRVTITCSASQGISGDLNWYQQKPGKAPKLLIYHTSQRHSDVPSRFSGSGSGTDFTLTISSLQPEDFATYYCQGYSKDLLTFGGGTKLEIKSSASTKGPSVFPLAPSSKSTSGGTAALGCLVKDYFPEPVTVSWNSGALTSGVHTFPAVLQSSGLYSLSSVVTVPSSSLGTQTYICNVNHKPSNTKVDKRVEPKSC

SEQ ID NO: 103 - protein, 451 aa, synthetic construct
QVQLVQSGAEVKKPGASVKVSCKASGYTFTNFYIHWVRQAPGQGLEWMGSIYPNYGITAYNQKFKDRVTMTVDTSTSTAYMELRSLRSDDTAVYYCARGYSYAMDYWGQGTTVTVSSASVAAPSVFIFPPSDEQLKSGTASVVCLLNNFYPREAKVQWKVDNALQSGNSQESVTEQDSKDSTYSLSSTLTLSKADYEKHKVYACEVTHQGLSSPVTKSFNRGECDKTHTCPPCPAPEAAGGPSVFLFPPKPKDTLMISRTPEVTCVVVDVSHEDPEVKFNWYVDGVEVHNAKTKPREEQYNSTYRVVSVLTVLHQDWLNGKEYKCKVSNKALAAPIEKTISKAKGQPREPQVYTLPPSREEMTKNQVSLTCLVKGFYPSDIAVEWESNGQPENNYKTTPPVLDSDGSFFLTSKLTVDKSRWQQGNVFSCSVMHEALHNHYTQKSLSLSPGK

SEQ ID NO: 104 - protein, 212 aa, synthetic construct
DIQMTQSPSSVSASVGDRVTITCSASQGISGDLNWYQQKPGKAPKLLIYHTSQLHSDVPSRFSGSGSGTDFTLTISSLQPEDFATYYCQGYSKDLLTFGGGTKLEIKSSASTKGPSVFPLAPSSKSTSGGTAALGCLVKDYFPEPVTVSWNSGALTSGVHTFPAVLQSSGLYSLSSVVTVPSSSLGTQTYICNVNHKPSNTKVDKRVEPKSC

SEQ ID NO: 105 - protein, 447 aa, synthetic construct
QVQLVQSGAEVKKPGASVKVSCKASGYTFTNFYIHWVRQAPGQGLEWMGRIYPNYGITAYNQKFKDRVTMTVDTSTSTAYMELRSLRSDDTAVYYCARGYSYAMDYWGQGTTVTVSSASTKGPSVFPLAPSSKSTSGGTAALGCLVKDYFPEPVTVSWNSGALTSGVHTFPAVLQSSGLYSLSSVVTVPSSSLGTQTYICNVNHKPSNTKVDKRVEPKSCDKTHTCPPCPAPEAAGGPSVFLFPPKPKDTLMISRTPEVTCVVVDVSHEDPEVKFNWYVDGVEVHNAKTKPREEQYNSTYRVVSVLTVLHQDWLNGKEYKCKVSNKALAAPIEKTISKAKGQPREPQVYTLPPSREEMTKNQVSLTCLVKGFYPSDIAVEWESNGQPENNYKTTPPVLDSDGSFFLTSKLTVDKSRWQQGNVFSCSVMHEALHNHYTQKSLSLSPGK

SEQ ID NO: 106 - protein, 214 aa, synthetic construct
DIQMTQSPSSVSASVGDRVTITCSASQGISGDLNWYQQKPGKAPKLLIYHTSQRHSDVPSRFSGSGSGTDFTLTISSLQPEDFATYYCQGYSKDLLTFGGGTKLEIKRTVAAPSVFIFPPSDEQLKSGTASVVCLLNNFYPREAKVQWKVDNALQSGNSQESVTEQDSKDSTYSLSSTLTLSKADYEKHKVYACEVTHQGLSSPVTKSFNRGEC

SEQ ID NO: 107 - protein, 841 aa, synthetic construct
AIRLTQSPSSFSASTGDRVTITCKASQSVDYGGGNFHLRPRDLISNINVIVLELKGSETTFMCEYADETATIVEFLNRWITFSQSIISTLTPTSSSTKKTQLQLEHLLLDLQMILNGINNYKNPKLTRMLTFKFYMPKKATELKHLQCLEEELKPLEEVLNLAQSKGGGGDSYMNWYQQKPGKAPKLLIYAASNLESGVPSRFSGSGSGTDFTLTISSLQSEDFATYYCQQSNEDPYTFGGGTKVEIKGGGGSGGGGSGGGGSEVQLVQSGAEVKKPGESLKISCKGSGYAFTNYLIEWVRQMPGKGLEWMGVINPGSGGTNYNEKFKGQVTISADKSISTAYLQWSSLKASDTAMYYCARWRGEGYYAYFDVWGQGTTVTVSSGGGGSGGGGSQVQLVQSGAEVKKPGASVKVSCKASGYTFTNFYIHWVRQAPGQGLEWMGRIYPNYGITAYNQKFKDRVTMTVDTSTSTAYMELRSLRSDDTAVYYCARGYSYAMDYWGQGTTVTVSSASTKGPSVFPLAPSSKSTSGGTAALGCLVKDYFPEPVTVSWNSGALTSGVHTFPAVLQSSGLYSLSSVVTVPSSSLGTQTYICNVNHKPSNTKVDKRVEPKSCDKTHTCPPCPAPEAAGGPSVFLFPPKPKDTLMISRTPEVTCVVVDVSHEDPEVKFNWYVDGVEVHNAKTKPREEQYNSTYRVVSVLTVLHQDWLNGKEYKCKVSNKALAAPIEKTISKAKGQPREPQVYTLPPSREEMTKNQVSLYCLVKGFYPSDIAVEWESNGQPENNYKTTPPVLDSDGSFFLYSKLTVDKSRWQQGNVFSCSVMHEALHNHYTQKSLSLSPGK

SEQ ID NO: 108 - protein, 447 aa, synthetic construct
QVQLVQSGAEVKKPGASVKVSCKASGYTFTNFYIHWVRQAPGQGLEWMGSIYPNYGITAYNQKFKDRVTMTVDTSTSTAYMELRSLRSDDTAVYYCARGYSYAMDYWGQGTTVTVSSASTKGPSVFPLAPSSKSTSGGTAALGCLVKDYFPEPVTVSWNSGALTSGVHTFPAVLQSSGLYSLSSVVTVPSSSLGTQTYICNVNHKPSNTKVDKRVEPKSCDKTHTCPPCPAPEAAGGPSVFLFPPKPKDTLMISRTPEVTCVVVDVSHEDPEVKFNWYVDGVEVHNAKTKPREEQYNSTYRVVSVLTVLHQDWLNGKEYKCKVSNKALAAPIEKTISKAKGQPREPQVYTLPPSREEMTKNQVSLTCLVKGFYPSDIAVEWESNGQPENNYKTTPPVLDSDGSFFLTSKLTVDKSRWQQGNVFSCSVMHEALHNHYTQKSLSLSPGK

SEQ ID NO: 109 - protein, 214 aa, synthetic construct
DIQMTQSPSSVSASVGDRVTITCSASQGISGDLNWYQQKPGKAPKLLIYHTSQLHSDVPSRFSGSGSGTDFTLTISSLQPEDFATYYCQGYSKDLLTFGGGTKLEIKRTVAAPSVFIFPPSDEQLKSGTASVVCLLNNFYPREAKVQWKVDNALQSGNSQESVTEQDSKDSTYSLSSTLTLSKADYEKHKVYACEVTHQGLSSPVTKSFNRGEC

SEQ ID NO: 110 - protein, 841 aa, synthetic construct
AIRLTQSPSSFSASTGDRVTITCKASQSVDYGGGNFHLRPRDLISNINVIVLELKGSETTFMCEYADETATIVEFLNRWITFSQSIISTLTPTSSSTKKTQLQLEHLLLDLQMILNGINNYKNPKLTRMLTFKFYMPKKATELKHLQCLEEELKPLEEVLNLAQSKGGGGDSYMNWYQQKPGKAPKLLIYAASNLESGVPSRFSGSGSGTDFTLTISSLQSEDFATYYCQQSNEDPYTFGGGTKVEIKGGGGSGGGGSGGGGSEVQLVQSGAEVKKPGESLKISCKGSGYAFTNYLIEWVRQMPGKGLEWMGVINPGSGGTNYNEKFKGQVTISADKSISTAYLQWSSLKASDTAMYYCARWRGEGYYAYFDVWGQGTTVTVSSGGGGSGGGGSQVQLVQSGAEVKKPGASVKVSCKASGYTFTNFYIHWVRQAPGQGLEWMGSIYPNYGITAYNQKFKDRVTMTVDTSTSTAYMELRSLRSDDTAVYYCARGYSYAMDYWGQGTTVTVSSASTKGPSVFPLAPSSKSTSGGTAALGCLVKDYFPEPVTVSWNSGALTSGVHTFPAVLQSSGLYSLSSVVTVPSSSLGTQTYICNVNHKPSNTKVDKRVEPKSCDKTHTCPPCPAPEAAGGPSVFLFPPKPKDTLMISRTPEVTCVVVDVSHEDPEVKFNWYVDGVEVHNAKTKPREEQYNSTYRVVSVLTVLHQDWLNGKEYKCKVSNKALAAPIEKTISKAKGQPREPQVYTLPPSREEMTKNQVSLYCLVKGFYPSDIAVEWESNGQPENNYKTTPPVLDSDGSFFLYSKLTVDKSRWQQGNVFSCSVMHEALHNHYTQKSLSLSPGK

SEQ ID NO: 111 - protein, 445 aa, synthetic construct
EVQLLESGGGLVQPGGSLRLSCAASGFTFSINAMTWVRQAPGKGLEWVSTISGSGFSTYYADSLKGRFTISRDNSKNTLYLQMNSLRAEDTAVYYCAKEVYGDYWGQGTLVTVSSASTKGPSVFPLAPSSKSTSGGTAALGCLVKDYFPEPVTVSWNSGALTSGVHTFPAVLQSSGLYSLSSVVTVPSSSLGTQTYICNVNHKPSNTKVDKRVEPKSCDKTHTCPPCPAPEAAGGPSVFLFPPKPKDTLMISRTPEVTCVVVDVSHEDPEVKFNWYVDGVEVHNAKTKPREEQYNSTYRVVSVLTVLHQDWLNGKEYKCKVSNKALAAPIEKTISKAKGQPREPQVCTLPPSREEMTKNQVSLSCAVKGFYPSDIAVEWESNGQPENNYKTTPPVLDSDGSFFLVSKLTVDKSRWQQGNVFSCSVMHEALHNHYTQKSLSLSPGK

SEQ ID NO: 112 - protein, 451 aa, synthetic construct
EVQLVQSGAEVKKPGESLKISCKGSGYAFTNYLIEWVRQMPGKGLEWMGVINPGSGGTNYNEKFKGQVTISADKSISTAYLQWSSLKASDTAMYYCARWRGEGYYAYFDVWGQGTTVTVSSASTKGPSVFPLAPSSKSTSGGTAALGCLVKDYFPEPVTVSWNSGALTSGVHTFPAVLQSSGLYSLSSVVTVPSSSLGTQTYICNVNHKPSNTKVDKRVEPKSCDKTHTCPPCPAPEAAGGPSVFLFPPKPKDTLMISRTPEVTCVVVDVSHEDPEVKFNWYVDGVEVHNAKTKPREEQYNSTYRVVSVLTVLHQDWLNGKEYKCKVSNKALAAPIEKTISKAKGQPREPQVYTLPPCREEMTKNQVSLWCLVKGFYPSDIAVEWESNGQPENNYKTTPPVLDSDGSFFLYSKLTVDKSRWQQGNVFSCSVMHEALHNHYTQKSLSLSPGK

SEQ ID NO: 113 - protein, 447 aa, synthetic construct
QVQLVQSGAEVKKPGASVKVSCKASGYTFTNFYIHWVRQAPGQGLEWMGRIYPNYGITAYNQKFKDRVTMTVDTSTSTAYMELRSLRSDDTAVYYCARGYSYAMDYWGQGTTVTVSSASTKGPSVFPLAPSSKSTSGGTAALGCLVKDYFPEPVTVSWNSGALTSGVHTFPAVLQSSGLYSLSSVVTVPSSSLGTQTYICNVNHKPSNTKVDKRVEPKSCDKTHTCPPCPAPEAAGGPSVFLFPPKPKDTLMISRTPEVTCVVVDVSHEDPEVKFNWYVDGVEVHNAKTKPREEQYNSTYRVVSVLTVLHQDWLNGKEYKCKVSNKALAAPIEKTISKAKGQPREPQVCTLPPSREEMTKNQVSLSCAVKGFYPSDIAVEWESNGQPENNYKTTPPVLDSDGSFFLVSKLTVDKSRWQQGNVFSCSVMHEALHNHYTQKSLSLSPGK

SEQ ID NO: 114 - protein, 841 aa, synthetic construct
AIRLTQSPSSFSASTGDRVTITCKASQSVDYGGGNFHLRPRDLISNINVIVLELKGSETTFMCEYADETATIVEFLNRWITFSQSIISTLTPTSSSTKKTQLQLEHLLLDLQMILNGINNYKNPKLTRMLTFKFYMPKKATELKHLQCLEEELKPLEEVLNLAQSKGGGGDSYMNWYQQKPGKAPKLLIYAASNLESGVPSRFSGSGSGTDFTLTISSLQSEDFATYYCQQSNEDPYTFGGGTKVEIKGGGGSGGGGSGGGGSEVQLVQSGAEVKKPGESLKISCKGSGYAFTNYLIEWVRQMPGKGLEWMGVINPGSGGTNYNEKFKGQVTISADKSISTAYLQWSSLKASDTAMYYCARWRGEGYYAYFDVWGQGTTVTVSSGGGGSGGGGSQVQLVQSGAEVKKPGASVKVSCKASGYTFTNFYIHWVRQAPGQGLEWMGRIYPNYGITAYNQKFKDRVTMTVDTSTSTAYMELRSLRSDDTAVYYCARGYSYAMDYWGQGTTVTVSSASTKGPSVFPLAPSSKSTSGGTAALGCLVKDYFPEPVTVSWNSGALTSGVHTFPAVLQSSGLYSLSSVVTVPSSSLGTQTYICNVNHKPSNTKVDKRVEPKSCDKTHTCPPCPAPEAAGGPSVFLFPPKPKDTLMISRTPEVTCVVVDVSHEDPEVKFNWYVDGVEVHNAKTKPREEQYNSTYRVVSVLTVLHQDWLNGKEYKCKVSNKALAAPIEKTISKAKGQPREPQVYTLPPCREEMTKNQVSLWCLVKGFYPSDIAVEWESNGQPENNYKTTPPVLDSDGSFFLYSKLTVDKSRWQQGNVFSCSVMHEALHNHYTQKSLSLSPGK

SEQ ID NO: 115 - protein, 447 aa, synthetic construct
QVQLVQSGAEVKKPGASVKVSCKASGYTFTNFYIHWVRQAPGQGLEWMGSIYPNYGITAYNQKFKDRVTMTVDTSTSTAYMELRSLRSDDTAVYYCARGYSYAMDYWGQGTTVTVSSASTKGPSVFPLAPSSKSTSGGTAALGCLVKDYFPEPVTVSWNSGALTSGVHTFPAVLQSSGLYSLSSVVTVPSSSLGTQTYICNVNHKPSNTKVDKRVEPKSCDKTHTCPPCPAPEAAGGPSVFLFPPKPKDTLMISRTPEVTCVVVDVSHEDPEVKFNWYVDGVEVHNAKTKPREEQYNSTYRVVSVLTVLHQDWLNGKEYKCKVSNKALAAPIEKTISKAKGQPREPQVCTLPPSREEMTKNQVSLSCAVKGFYPSDIAVEWESNGQPENNYKTTPPVLDSDGSFFLVSKLTVDKSRWQQGNVFSCSVMHEALHNHYTQKSLSLSPGK

SEQ ID NO: 116 - protein, 841 aa, synthetic construct
AIRLTQSPSSFSASTGDRVTITCKASQSVDYGGGNFHLRPRDLISNINVIVLELKGSETTFMCEYADETATIVEFLNRWITFSQSIISTLTPTSSSTKKTQLQLEHLLLDLQMILNGINNYKNPKLTRMLTFKFYMPKKATELKHLQCLEEELKPLEEVLNLAQSKGGGGDSYMNWYQQKPGKAPKLLIYAASNLESGVPSRFSGSGSGTDFTLTISSLQSEDFATYYCQQSNEDPYTFGGGTKVEIKGGGGSGGGGSGGGGSEVQLVQSGAEVKKPGESLKISCKGSGYAFTNYLIEWVRQMPGKGLEWMGVINPGSGGTNYNEKFKGQVTISADKSISTAYLQWSSLKASDTAMYYCARWRGEGYYAYFDVWGQGTTVTVSSGGGGSGGGGSQVQLVQSGAEVKKPGASVKVSCKASGYTFTNFYIHWVRQAPGQGLEWMGSIYPNYGITAYNQKFKDRVTMTVDTSTSTAYMELRSLRSDDTAVYYCARGYSYAMDYWGQGTTVTVSSASTKGPSVFPLAPSSKSTSGGTAALGCLVKDYFPEPVTVSWNSGALTSGVHTFPAVLQSSGLYSLSSVVTVPSSSLGTQTYICNVNHKPSNTKVDKRVEPKSCDKTHTCPPCPAPEAAGGPSVFLFPPKPKDTLMISRTPEVTCVVVDVSHEDPEVKFNWYVDGVEVHNAKTKPREEQYNSTYRVVSVLTVLHQDWLNGKEYKCKVSNKALAAPIEKTISKAKGQPREPQVYTLPPCREEMTKNQVSLWCLVKGFYPSDIAVEWESNGQPENNYKTTPPVLDSDGSFFLYSKLTVDKSRWQQGNVFSCSVMHEALHNHYTQKSLSLSPGK

SEQ ID NO: 117 - protein, 451 aa, synthetic construct
QVQLVQSGAEVKKPGASVKVSCKASGYTFTNFYIHWVRQAPGQGLEWMGSIYPNYGITAYNQKFKDRVTMTVDTSTSTAYMELRSLRSDDTAVYYCARGYSYAMDYWGQGTTVTVSSASVAAPSVFIFPPSDEQLKSGTASVVCLLNNFYPREAKVQWKVDNALQSGNSQESVTEQDSKDSTYSLSSTLTLSKADYEKHKVYACEVTHQGLSSPVTKSFNRGECDKTHTCPPCPAPEAAGGPSVFLFPPKPKDTLMISRTPEVTCVVVDVSHEDPEVKFNWYVDGVEVHNAKTKPREEQYNSTYRVVSVLTVLHQDWLNGKEYKCKVSNKALAAPIEKTISKAKGQPREPQVCTLPPSREEMTKNQVSLSCAVKGFYPSDIAVEWESNGQPENNYKTTPPVLDSDGSFFLVSKLTVDKSRWQQGNVFSCSVMHEALHNHYTQKSLSLSPGK

SEQ ID NO: 118 - protein, 10 aa, synthetic construct
GFTFSINAMT

SEQ ID NO: 119 - protein, 18 aa, synthetic construct
TISGSGFSTYYADSLKGR

SEQ ID NO: 120 - protein, 6 aa, synthetic construct
EVYGDY

SEQ ID NO: 121 - protein, 14 aa, synthetic construct
  VARIANT 3: note = X = N, S,Q or A
  REGION 11..12: note = XX = NS, QS, SS or NA
SGXSSNIGSXXXVF

SEQ ID NO: 122 - protein, 7 aa, synthetic construct
SNNQRPS

SEQ ID NO: 123 - protein, 12 aa, synthetic construct
AAWDDSLSIWVF

SEQ ID NO: 124 - protein, 13 aa, synthetic construct
SGASSNIGSQSVF

SEQ ID NO: 125 - protein, 13 aa, synthetic construct
SGASSNIGSSSVF

SEQ ID NO: 126 - protein, 13 aa, synthetic construct
SGASSNIGSNAVF

SEQ ID NO: 127 - protein, 5 aa, synthetic construct
NFYIH

SEQ ID NO: 128 - protein, 17 aa, synthetic construct
RIYPNYGITAYNQKFKD

SEQ ID NO: 129 - protein, 8 aa, synthetic construct
GYSYAMDY

SEQ ID NO: 130 - protein, 11 aa, synthetic construct
SASQGISGDLN

SEQ ID NO: 131 - protein, 7 aa, synthetic construct
HTSQRHS

SEQ ID NO: 132 - protein, 9 aa, synthetic construct
QGYSKDLLT

SEQ ID NO: 133 - protein, 17 aa, synthetic construct
SIYPNYGITAYNQKFKD

SEQ ID NO: 134 - protein, 7 aa, synthetic construct
HTSQLHS

SEQ ID NO: 135 - protein, 10 aa, synthetic construct
GFTFSISAMT

SEQ ID NO: 136 - protein, 17 aa, synthetic construct
TISGSGGSTYYSDSVKG

SEQ ID NO: 137 - protein, 11 aa, synthetic construct
SGSSSNIGSNS

SEQ ID NO: 138 - protein, 10 aa, synthetic construct
GFTFSTYAMS

SEQ ID NO: 139 - protein, 17 aa, synthetic construct
TISGTGYSTYFADSVKG

SEQ ID NO: 140 - protein, 11 aa, synthetic construct
SGRSSNIGSNS

SEQ ID NO: 141 - protein, 11 aa, synthetic construct
AAWDDSLSGWV

SEQ ID NO: 142 - protein, 8 aa, synthetic construct
GFTFSSYS

SEQ ID NO: 143 - protein, 17 aa, synthetic construct
FISSSSPTLYYADSVKG

SEQ ID NO: 144 - protein, 10 aa, synthetic construct
ARQGLTPFDY

SEQ ID NO: 145 - protein, 11 aa, synthetic construct
RASQSVSSYLA

SEQ ID NO: 146 - protein, 7 aa, synthetic construct
GASTRAT

SEQ ID NO: 147 - protein, 9 aa, synthetic construct
QQYNNWPYT

SEQ ID NO: 148 - protein, 10 aa, synthetic construct
GFTFSNYGMH

SEQ ID NO: 149 - protein, 17 aa, synthetic construct
VIWYDGSKKYYADSVKG

SEQ ID NO: 150 - protein, 4 aa, synthetic construct
NSGH

SEQ ID NO: 151 - protein, 17 aa, synthetic construct
RSSQSLLDSDDGNTYLD

SEQ ID NO: 152 - protein, 7 aa, synthetic construct
TLSYRAS

SEQ ID NO: 153 - protein, 9 aa, synthetic construct
MQCIEFPHT

SEQ ID NO: 154 - protein, 10 aa, synthetic construct
GFTFSSYSMN

SEQ ID NO: 155 - protein, 17 aa, synthetic construct
YITSSSNTMYYADSVKG

SEQ ID NO: 156 - protein, 8 aa, synthetic construct
IVGAPFDY

SEQ ID NO: 157 - protein, 11 aa, synthetic construct
RASQSVSSSLA

SEQ ID NO: 158 - protein, 9 aa, synthetic construct
QQYNNWPFT

SEQ ID NO: 159 - protein, 10 aa, synthetic construct
GYTFTSYFMH

SEQ ID NO: 160 - protein, 17 aa, synthetic construct
LINPDGGNTDYAQKFQG

SEQ ID NO: 161 - protein, 18 aa, synthetic construct
DGNYYDSSGYYYPDAFDI

SEQ ID NO: 162 - protein, 11 aa, synthetic construct
QGDSLRRFYAS

SEQ ID NO: 163 - protein, 7 aa, synthetic construct
GKDNRPS

SEQ ID NO: 164 - protein, 11 aa, synthetic construct
NSRDSSGTHVV

SEQ ID NO: 165 - protein, 17 aa, synthetic construct
  VARIANT 1: note = X = R or S
XIYPNYGITAYNQKFKD

SEQ ID NO: 166 - protein, 7 aa, synthetic construct
  VARIANT 5: note = X = L or R
HTSQXHS

SEQ ID NO: 167 - protein, 248 aa, synthetic construct; identical to SEQ ID NO: 27